European Patent Application EP 4 342 999 A2, published March 27, 2024. Title: COMPOSITIONS, KITS AND METHODS FOR ISOLATING TARGET POLYNUCLEOTIDES. Applicant: DNAe DIAGNOSTICS LIMITED. Application EP. The sequence listing filed with the application follows.

SEQUENCE LISTING (39 sequences)

SEQ ID NO: 1 - DNA, 24 bp, Escherichia coli
  source 1..24: mol_type = genomic DNA
gtatcagcgcgaagtctttatacc

SEQ ID NO: 2 - DNA, 24 bp, Escherichia coli
  source 1..24: mol_type = genomic DNA
ggcaataacatacggagtgacatc

SEQ ID NO: 3 - DNA, 169 bp, Escherichia coli
  source 1..169: mol_type = genomic DNA
gtatcagcgcgaagtctttataccgaaaggttgggcgggccagcgtattgtactgcgtttcgatgcggtcactcattacggcaaagtgtgggtaaataatcaggaagtgatggagcatcagggcggctatacgccatttgaagccgatgtcactccgtatgttattgcc

SEQ ID NO: 4 - DNA, 41 bp, synthetic construct
  misc_feature >41: note = Hexaethylene Glycol (HEG) internal spacer followed by SEQ ID NO: 37
  source 1..41: mol_type = other DNA
aaaaaaaaaaaaaaaaaaaaaaaaaaaaaaaaaaacctcta

SEQ ID NO: 5 - DNA, 22 bp, synthetic construct
  source 1..22: mol_type = other DNA
agacgcaagctactggtgattt

SEQ ID NO: 6 - DNA, 30 bp, synthetic construct
  source 1..30: mol_type = other DNA
ggcaataacatacggagtgacatcggcttc

SEQ ID NO: 7 - DNA, 20 bp, synthetic construct
  misc_feature >20: note = 3' Biotin
  source 1..20: mol_type = other DNA
tttttttttttttttttttt

SEQ ID NO: 8 - DNA, 29 bp, synthetic construct
  misc_feature >29: note = 3' IowaBlack
  source 1..29: mol_type = other DNA
  misc_feature <1: note = 5' FAM
tagccgccctgatgctccatcacttcctg

SEQ ID NO: 9 - DNA, 20 bp, synthetic construct
  source 1..20: mol_type = other DNA
agacgcaagctactggtgat

SEQ ID NO: 10 - DNA, 22 bp, Enterococcus faecium
  source 1..22: mol_type = genomic DNA
ggctgcgatattcaaagctcag

SEQ ID NO: 11 - DNA, 19 bp, Enterococcus faecium
  source 1..19: mol_type = genomic DNA
ctgaacgcgccggcttaac

SEQ ID NO: 12 - DNA, 166 bp, Enterococcus faecium
  source 1..166: mol_type = genomic DNA
ggctgcgatattcaaagctcagcaatttgtatggacaaatcgttgacatacatcgttgcgaaaaatgctgggatagctactcccgccttttgggttattaataaagatgataggccggtggcagctacgtttacctatcctgtttttgttaagccggcgcgttcag

SEQ ID NO: 13 - DNA, 20 bp, synthetic construct
  misc_feature >20: note = Hexaethylene Glycol (HEG) internal spacer followed by SEQ ID NO: 38
  source 1..20: mol_type = other DNA
aaaaaaaaaaaaaaaaaaaa

SEQ ID NO: 14 - DNA, 38 bp, synthetic construct
  source 1..38: mol_type = other DNA
ctcctctggcaccgtgctgccttggcttcattgtggtc

SEQ ID NO: 15 - DNA, 19 bp, synthetic construct
  source 1..19: mol_type = other DNA
ctgaacgcgccggcttaac

SEQ ID NO: 16 - DNA, 25 bp, synthetic construct
  source 1..25: mol_type = other DNA
  modified_base 25: mod_base = OTHER; note = inverted T nucleotide which serves as a blocking moiety
cggtgccagaggagttttttttttt

SEQ ID NO: 17 - DNA, 14 bp, synthetic construct
  source 1..14: mol_type = other DNA
cggtgccagaggag

SEQ ID NO: 18 - DNA, 10 bp, synthetic construct
  source 1..10: mol_type = other DNA
tttttttttt

SEQ ID NO: 19 - DNA, 20 bp, synthetic construct
  misc_feature >20: note = 3' Biotin
  source 1..20: mol_type = other DNA
tttttttttttttttttttt

SEQ ID NO: 20 - DNA, 26 bp, synthetic construct
  source 1..26: mol_type = other DNA
ttgtatggacaaatcgttgacataca

SEQ ID NO: 21 - DNA, 28 bp, synthetic construct
  misc_feature >28: note = 3' IowaBlack
  source 1..28: mol_type = other DNA
  misc_feature <1: note = 5' FAM
tgctgggatagctactcccgccttttgg

SEQ ID NO: 22 - DNA, 19 bp, synthetic construct
  source 1..19: mol_type = other DNA
accgtgctgccttggcttc

SEQ ID NO: 23 - DNA, 22 bp, Enterococcus faecium
  source 1..22: mol_type = genomic DNA
ggctgcgatattcaaagctcag

SEQ ID NO: 24 - DNA, 19 bp, Enterococcus faecium
  source 1..19: mol_type = genomic DNA
ctgaacgcgccggcttaac

SEQ ID NO: 25 - DNA, 166 bp, Enterococcus faecium; identical to SEQ ID NO: 12
  source 1..166: mol_type = genomic DNA

SEQ ID NO: 26 - DNA, 20 bp, synthetic construct
  misc_feature >20: note = Hexaethylene Glycol (HEG) internal spacer followed by SEQ ID NO: 39
  source 1..20: mol_type = other DNA
aaaaaaaaaaaaaaaaaaaa

SEQ ID NO: 27 - DNA, 38 bp, synthetic construct; identical to SEQ ID NO: 14
  source 1..38: mol_type = other DNA

SEQ ID NO: 28 - DNA, 19 bp, synthetic construct
  source 1..19: mol_type = other DNA
gtagctgccaccggcctat

SEQ ID NO: 29 - DNA, 25 bp, synthetic construct
  source 1..25: mol_type = other DNA
  modified_base 25: mod_base = OTHER; note = inverted T nucleotide which serves as a blocking moiety
cggtgccagaggagttttttttttt

SEQ ID NO: 30 - DNA, 14 bp, synthetic construct
  source 1..14: mol_type = other DNA
cggtgccagaggag

SEQ ID NO: 31 - DNA, 10 bp, synthetic construct
  source 1..10: mol_type = other DNA
tttttttttt

SEQ ID NO: 32 - DNA, 47 bp, synthetic construct
  source 1..47: mol_type = other DNA
aaaacgagacatgccgagcatccgcggctgcgatattcaaagctcag

SEQ ID NO: 33 - DNA, 20 bp, synthetic construct
  misc_feature >20: note = 3' Biotin
  source 1..20: mol_type = other DNA
tttttttttttttttttttt

SEQ ID NO: 34 - DNA, 22 bp, synthetic construct
  source 1..22: mol_type = other DNA
aaaacgagacatgccgagcatc

SEQ ID NO: 35 - DNA, 28 bp, synthetic construct
  misc_feature >28: note = 3' IowaBlack
  source 1..28: mol_type = other DNA
  misc_feature <1: note = 5' FAM
tgctgggatagctactcccgccttttgg

SEQ ID NO: 36 - DNA, 19 bp, synthetic construct
  source 1..19: mol_type = other DNA
accgtgctgccttggcttc

SEQ ID NO: 37 - DNA, 87 bp, synthetic construct
  source 1..87: mol_type = other DNA
  misc_feature <1: note = Hexaethylene Glycol (HEG) internal spacer preceded by SEQ ID NO: 4
tttttttttttttttttttttttttttttttttttagacgcaagctactggtgatttggcaataacatacggagtgacatcggcttc

SEQ ID NO: 38 - DNA, 57 bp, synthetic construct
  source 1..57: mol_type = other DNA
  misc_feature <1: note = Hexaethylene Glycol (HEG) internal spacer preceded by SEQ ID NO: 13
ctcctctggcaccgtgctgccttggcttcattgtggtcctgaacgcgccggcttaac

SEQ ID NO: 39 - DNA, 57 bp, synthetic construct
  source 1..57: mol_type = other DNA
  misc_feature <1: note = Hexaethylene Glycol (HEG) internal spacer preceded by SEQ ID NO: 26
ctcctctggcaccgtgctgccttggcttcattgtggtcgtagctgccaccggcctat